European Patent Application EP 4 410 986 A2, published August 7, 2024. Title: CELLS, VERTEBRATES, POPULATIONS & METHODS. Applicant: Kymab Limited. Application EP. The sequence listing filed with the application follows.

SEQUENCE LISTING (1 sequence)

SEQ ID NO: 1 - protein, 107 aa, Homo sapiens
YVLTQPPSVSVAPGETARITCGGDNIGRKSVYWYQQKSGQAPVLVIYYDSDRPSGIPERFSGSNSGNTATLTISRVEAGDEADYYCQVWDGSSDHWVFGGGTKLTVL